European Patent Application EP 4 458 863 A1, published November 6, 2024. Title: Fusion Protein of GLP-1/GDF15 and use thereof. Applicant: 广东东阳光药业有限公司. Application CN. The sequence listing filed with the application follows.

SEQUENCE LISTING (130 sequences)

SEQ ID NO: 1 - protein, 37 aa, synthetic construct
HDEFERHAEGTFTSDVSSYLEGQAAKEFIAWLVKGRG

SEQ ID NO: 2 - protein, 31 aa, synthetic construct
HAEGTFTSDVSSYLEGQAAKEFIAWLVKGRG

SEQ ID NO: 3 - protein, 36 aa, synthetic construct
HDEFERHAEGTFTSDVSSYLEGQAAKEFIAWLVKGR

SEQ ID NO: 4 - protein, 30 aa, synthetic construct
HAEGTFTSDVSSYLEGQAAKEFIAWLVKGR

SEQ ID NO: 5 - protein, 31 aa, synthetic construct
HGEGTFTSDVSSYLEEQAAKEFIAWLVKGGG

SEQ ID NO: 6 - protein, 31 aa, synthetic construct
HGEGTFTSDVSSYLEEQAAKEFIEWLVKGGG

SEQ ID NO: 7 - protein, 31 aa, synthetic construct
HGEGTFTSDVSSYLEEQAAKEFIQWLVKGGG

SEQ ID NO: 8 - protein, 31 aa, synthetic construct
HGEGTFTSDVSSYLEEQAAKEFVQWLVKGGG

SEQ ID NO: 9 - protein, 210 aa, synthetic construct
GPSVFLFPPKPKDTLMISRTPEVTCVVVDVSQEDPEVQFNWYVDGVEVHNAKTKPREEQFNSTYRVVSVLTVLHQDWLNGKEYKCKVSNKGLPSSIEKTISKAKGQPREPQVYTLPPSQEEMTKNQVSLTCLVKGFYPSDIAVEWESNGQPENNYKTTPPVLDSDGSFFLYSRLTVDKSRWQEGNVFSCSVMHEALHNHYTQKSLSLSLG

SEQ ID NO: 10 - protein, 211 aa, synthetic construct
GGPSVFLFPPKPKDTLMISRTPEVTCVVVDVSQEDPEVQFNWYVDGVEVHNAKTKPREEQFNSTYRVVSVLTVLHQDWLNGKEYKCKVSNKGLPSSIEKTISKAKGQPREPQVYTLPPSQEEMTKNQVSLTCLVKGFYPSDIAVEWESNGQPENNYKTTPPVLDSDGSFFLYSRLTVDKSRWQEGNVFSCSVMHEALHNHYTQKSLSLSLG

SEQ ID NO: 11 - protein, 214 aa, synthetic construct
EAAGGPSVFLFPPKPKDTLMISRTPEVTCVVVDVSQEDPEVQFNWYVDGVEVHNAKTKPREEQFNSTYRVVSVLTVLHQDWLNGKEYKCKVSNKGLPSSIEKTISKAKGQPREPQVYTLPPSQEEMTKNQVSLTCLVKGFYPSDIAVEWESNGQPENNYKTTPPVLDSDGSFFLYSRLTVDKSRWQEGNVFSCSVMHEALHNHYTQKSLSLSLG

SEQ ID NO: 12 - protein, 216 aa, synthetic construct
APEAAGGPSVFLFPPKPKDTLMISRTPEVTCVVVDVSQEDPEVQFNWYVDGVEVHNAKTKPREEQFNSTYRVVSVLTVLHQDWLNGKEYKCKVSNKGLPSSIEKTISKAKGQPREPQVYTLPPSQEEMTKNQVSLTCLVKGFYPSDIAVEWESNGQPENNYKTTPPVLDSDGSFFLYSRLTVDKSRWQEGNVFSCSVMHEALHNHYTQKSLSLSLG

SEQ ID NO: 13 - protein, 210 aa, synthetic construct
GPSVFLFPPKPKDTLMISRTPEVTCVVVDVSQEDPEVQFNWYVDGVEVHNAKTKPREEQFNSTYRVVSVLTVLHQDWLNGKEYKCKVSNKGLPSSIEKTISKAKGQPREPQVYTLPPSQEEMTKNQVSLTCLVKGFYPSDIAVEWESNGQPENNYKTTPPVLDSDGSFFLYSRLTVDKSRWQEGNVFSCSVMHEALHNHYTQESLSLSLG

SEQ ID NO: 14 - protein, 211 aa, synthetic construct
GGPSVFLFPPKPKDTLMISRTPEVTCVVVDVSQEDPEVQFNWYVDGVEVHNAKTKPREEQFNSTYRVVSVLTVLHQDWLNGKEYKCKVSNKGLPSSIEKTISKAKGQPREPQVYTLPPSQEEMTKNQVSLTCLVKGFYPSDIAVEWESNGQPENNYKTTPPVLDSDGSFFLYSRLTVDKSRWQEGNVFSCSVMHEALHNHYTQESLSLSLG

SEQ ID NO: 15 - protein, 214 aa, synthetic construct
EAAGGPSVFLFPPKPKDTLMISRTPEVTCVVVDVSQEDPEVQFNWYVDGVEVHNAKTKPREEQFNSTYRVVSVLTVLHQDWLNGKEYKCKVSNKGLPSSIEKTISKAKGQPREPQVYTLPPSQEEMTKNQVSLTCLVKGFYPSDIAVEWESNGQPENNYKTTPPVLDSDGSFFLYSRLTVDKSRWQEGNVFSCSVMHEALHNHYTQESLSLSLG

SEQ ID NO: 16 - protein, 216 aa, synthetic construct
APEAAGGPSVFLFPPKPKDTLMISRTPEVTCVVVDVSQEDPEVQFNWYVDGVEVHNAKTKPREEQFNSTYRVVSVLTVLHQDWLNGKEYKCKVSNKGLPSSIEKTISKAKGQPREPQVYTLPPSQEEMTKNQVSLTCLVKGFYPSDIAVEWESNGQPENNYKTTPPVLDSDGSFFLYSRLTVDKSRWQEGNVFSCSVMHEALHNHYTQESLSLSLG

SEQ ID NO: 17 - protein, 210 aa, synthetic construct
GPSVFLFPPKPKDTLMISRTPEVTCVVVDVSQEDPEVQFNWYVDGVEVHNAKTKPREEQFNSTYRVVSVLTVLHQDWLNGKEYKCKVSNKGLPSSIEKTISKAKGQPREPQVYTLPPSQEEMTKNQVSLTCLVKGFYPSDIAVEWESNGQPENNYKTTPPVLDSDGSFFLYSRLTVDKSRWQEGNVFSCSVMHEALHNHYTQDSLSLSLG

SEQ ID NO: 18 - protein, 211 aa, synthetic construct
GGPSVFLFPPKPKDTLMISRTPEVTCVVVDVSQEDPEVQFNWYVDGVEVHNAKTKPREEQFNSTYRVVSVLTVLHQDWLNGKEYKCKVSNKGLPSSIEKTISKAKGQPREPQVYTLPPSQEEMTKNQVSLTCLVKGFYPSDIAVEWESNGQPENNYKTTPPVLDSDGSFFLYSRLTVDKSRWQEGNVFSCSVMHEALHNHYTQDSLSLSLG

SEQ ID NO: 19 - protein, 214 aa, synthetic construct
EAAGGPSVFLFPPKPKDTLMISRTPEVTCVVVDVSQEDPEVQFNWYVDGVEVHNAKTKPREEQFNSTYRVVSVLTVLHQDWLNGKEYKCKVSNKGLPSSIEKTISKAKGQPREPQVYTLPPSQEEMTKNQVSLTCLVKGFYPSDIAVEWESNGQPENNYKTTPPVLDSDGSFFLYSRLTVDKSRWQEGNVFSCSVMHEALHNHYTQDSLSLSLG

SEQ ID NO: 20 - protein, 216 aa, synthetic construct
APEAAGGPSVFLFPPKPKDTLMISRTPEVTCVVVDVSQEDPEVQFNWYVDGVEVHNAKTKPREEQFNSTYRVVSVLTVLHQDWLNGKEYKCKVSNKGLPSSIEKTISKAKGQPREPQVYTLPPSQEEMTKNQVSLTCLVKGFYPSDIAVEWESNGQPENNYKTTPPVLDSDGSFFLYSRLTVDKSRWQEGNVFSCSVMHEALHNHYTQDSLSLSLG

SEQ ID NO: 21 - protein, 210 aa, synthetic construct
GPSVFLFPPKPKDTLMISRTPEVTCVVVDVSQEDPEVQFNWYVDGVEVHNAKTKPREEQFNSTYRVVSVLTVLHQDWLNGKEYKCKVSNKGLPSSIEKTISKAKGQPREPQVYTLPPSQKEMTKNQVSLTCLVKGFYPSDIAVEWESNGQPENNYKTTPPVLDSDGSFFLYSRLTVDKSRWQEGNVFSCSVMHEALHNHYTQKSLSLSLG

SEQ ID NO: 22 - protein, 211 aa, synthetic construct
GGPSVFLFPPKPKDTLMISRTPEVTCVVVDVSQEDPEVQFNWYVDGVEVHNAKTKPREEQFNSTYRVVSVLTVLHQDWLNGKEYKCKVSNKGLPSSIEKTISKAKGQPREPQVYTLPPSQKEMTKNQVSLTCLVKGFYPSDIAVEWESNGQPENNYKTTPPVLDSDGSFFLYSRLTVDKSRWQEGNVFSCSVMHEALHNHYTQKSLSLSLG

SEQ ID NO: 23 - protein, 214 aa, synthetic construct
EAAGGPSVFLFPPKPKDTLMISRTPEVTCVVVDVSQEDPEVQFNWYVDGVEVHNAKTKPREEQFNSTYRVVSVLTVLHQDWLNGKEYKCKVSNKGLPSSIEKTISKAKGQPREPQVYTLPPSQKEMTKNQVSLTCLVKGFYPSDIAVEWESNGQPENNYKTTPPVLDSDGSFFLYSRLTVDKSRWQEGNVFSCSVMHEALHNHYTQKSLSLSLG

SEQ ID NO: 24 - protein, 216 aa, synthetic construct
APEAAGGPSVFLFPPKPKDTLMISRTPEVTCVVVDVSQEDPEVQFNWYVDGVEVHNAKTKPREEQFNSTYRVVSVLTVLHQDWLNGKEYKCKVSNKGLPSSIEKTISKAKGQPREPQVYTLPPSQKEMTKNQVSLTCLVKGFYPSDIAVEWESNGQPENNYKTTPPVLDSDGSFFLYSRLTVDKSRWQEGNVFSCSVMHEALHNHYTQKSLSLSLG

SEQ ID NO: 25 - protein, 210 aa, synthetic construct
GPSVFLFPPKPKDTLMISRTPEVTCVVVDVSQEDPEVQFNWYVDGVEVHNAKTKPREEQFNSTYRVVSVLTVLHQDWLNGKEYKCKVSNKGLPSSIEKTISKAKGQPREPQVYTLPPSQREMTKNQVSLTCLVKGFYPSDIAVEWESNGQPENNYKTTPPVLDSDGSFFLYSRLTVDKSRWQEGNVFSCSVMHEALHNHYTQKSLSLSLG

SEQ ID NO: 26 - protein, 211 aa, synthetic construct
GGPSVFLFPPKPKDTLMISRTPEVTCVVVDVSQEDPEVQFNWYVDGVEVHNAKTKPREEQFNSTYRVVSVLTVLHQDWLNGKEYKCKVSNKGLPSSIEKTISKAKGQPREPQVYTLPPSQREMTKNQVSLTCLVKGFYPSDIAVEWESNGQPENNYKTTPPVLDSDGSFFLYSRLTVDKSRWQEGNVFSCSVMHEALHNHYTQKSLSLSLG

SEQ ID NO: 27 - protein, 214 aa, synthetic construct
EAAGGPSVFLFPPKPKDTLMISRTPEVTCVVVDVSQEDPEVQFNWYVDGVEVHNAKTKPREEQFNSTYRVVSVLTVLHQDWLNGKEYKCKVSNKGLPSSIEKTISKAKGQPREPQVYTLPPSQREMTKNQVSLTCLVKGFYPSDIAVEWESNGQPENNYKTTPPVLDSDGSFFLYSRLTVDKSRWQEGNVFSCSVMHEALHNHYTQKSLSLSLG

SEQ ID NO: 28 - protein, 216 aa, synthetic construct
APEAAGGPSVFLFPPKPKDTLMISRTPEVTCVVVDVSQEDPEVQFNWYVDGVEVHNAKTKPREEQFNSTYRVVSVLTVLHQDWLNGKEYKCKVSNKGLPSSIEKTISKAKGQPREPQVYTLPPSQREMTKNQVSLTCLVKGFYPSDIAVEWESNGQPENNYKTTPPVLDSDGSFFLYSRLTVDKSRWQEGNVFSCSVMHEALHNHYTQKSLSLSLG

SEQ ID NO: 29 - protein, 214 aa, synthetic construct
EAAGGPSVFLFPPKPKDTLMISRTPEVTCVVVDVSQEDPEVQFNWYVDGVEVHNAKTKPREEQFNSTYRVVSVLTVLHQDWLNGKEYKCKVSNKGLPSSIEKTISKAKGQPREPQVYTLPPSQEEMTKNQVSLTCLVKGFYPSDIAVEWESNGQPENNYKTTPPVLDSDGSFFLYSRLTVDKSRWQEGNVFSCSVMHEALHNHYTQQSLSLSLG

SEQ ID NO: 30 - protein, 216 aa, synthetic construct
APEAAGGPSVFLFPPKPKDTLMISRTPEVTCVVVDVSQEDPEVQFNWYVDGVEVHNAKTKPREEQFNSTYRVVSVLTVLHQDWLNGKEYKCKVSNKGLPSSIEKTISKAKGQPREPQVYTLPPSQEEMTKNQVSLTCLVKGFYPSDIAVEWESNGQPENNYKTTPPVLDSDGSFFLYSRLTVDKSRWQEGNVFSCSVMHEALHNHYTQQSLSLSLG

SEQ ID NO: 31 - protein, 216 aa, synthetic construct
APEAAGGPSVFLFPPKPKDTLMISRTPEVTCVVVDVSQEDPEVQFNWYVDGVEVHNAKTKPREEQFNSTYRVVSVLTVLHQDWLNGKEYKCKVSNKGLPSSIEKTISKAKGQPREPQVYTLPPSQEEMTKNQVSLTCLVKGFYPSDIAVEWESNGQPENNYKTTPPVLDSDGSFFLYSRLTVDKSRWQEGNVFSCSVMHEALHNHYTQNSLSLSLG

SEQ ID NO: 32 - protein, 216 aa, synthetic construct
APEAAGGPSVFLFPPKPKDTLMISRTPEVTCVVVDVSQEDPEVQFNWYVDGVEVHNAKTKPREEQFNSTYRVVSVLTVLHQDWLNGKEYKCKVSNKGLPSSIEKTISKAKGQPREPQVYTLPPSQEEMTKNQVSLTCLVKGFYPSDIAVEWESNGQPENNYKTTPPVLDSDGSFFLYSRLTVDKSRWQEGNVFSCSVMHEALHNHYTQASLSLSLG

SEQ ID NO: 33 - protein, 216 aa, synthetic construct
APEAAGGPSVFLFPPKPKDTLMISRTPEVTCVVVDVSQEDPEVQFNWYVDGVEVHNAKTKPREEQFNSTYRVVSVLTVLHQDWLNGKEYKCKVSNKGLPSSIEKTISKAKGQPREPQVYTLPPSQQEMTKNQVSLTCLVKGFYPSDIAVEWESNGQPENNYKTTPPVLDSDGSFFLYSRLTVDKSRWQEGNVFSCSVMHEALHNHYTQKSLSLSLG

SEQ ID NO: 34 - protein, 216 aa, synthetic construct
APEAAGGPSVFLFPPKPKDTLMISRTPEVTCVVVDVSQEDPEVQFNWYVDGVEVHNAKTKPREEQFNSTYRVVSVLTVLHQDWLNGKEYKCKVSNKGLPSSIEKTISKAKGQPREPQVYTLPPSQNEMTKNQVSLTCLVKGFYPSDIAVEWESNGQPENNYKTTPPVLDSDGSFFLYSRLTVDKSRWQEGNVFSCSVMHEALHNHYTQKSLSLSLG

SEQ ID NO: 35 - protein, 216 aa, synthetic construct
APEAAGGPSVFLFPPKPKDTLMISRTPEVTCVVVDVSQEDPEVQFNWYVDGVEVHNAKTKPREEQFNSTYRVVSVLTVLHQDWLNGKEYKCKVSNKGLPSSIEKTISKAKGQPREPQVYTLPPSQAEMTKNQVSLTCLVKGFYPSDIAVEWESNGQPENNYKTTPPVLDSDGSFFLYSRLTVDKSRWQEGNVFSCSVMHEALHNHYTQKSLSLSLG

SEQ ID NO: 36 - protein, 229 aa, synthetic construct
AESKYGPPCPPCPAPEAAGGPSVFLFPPKPKDTLMISRTPEVTCVVVDVSQEDPEVQFNWYVDGVEVHNAKTKPREEQFNSTYRVVSVLTVLHQDWLNGKEYKCKVSNKGLPSSIEKTISKAKGQPREPQVYTLPPSQEEMTKNQVSLTCLVKGFYPSDIAVEWESNGQPENNYKTTPPVLDSDGSFFLYSRLTVDKSRWQEGNVFSCSVMHEALHNHYTQESLSLSLG

SEQ ID NO: 37 - protein, 216 aa, synthetic construct
APEAAGGPSVFLFPPKPKDTLMISRTPEVTCVVVDVSHEDPEVKFNWYVDGVEVHNAKTKPREEQYNSTYRVVSVLTVLHQDWLNGKEYKCKVSNKALPAPIEKTISKAKGQPREPQVYTLPPSRDELTKNQVSLTCLVKGFYPSDIAVEWESNGQPENNYKTTPPVLDSDGSFFLYSKLTVDKSRWQQGNVFSCSVMHEALHNHYTQESLSLSPG

SEQ ID NO: 38 - protein, 112 aa, synthetic construct
ARNGDHCPLGPGRCCRLHTVRASLEDLGWADWVLSPREVQVTMCIGACPSQFRAANMHAQIKTSLHRLKPDTVPAPCCVPASYNPMVLIQKTDTGVSLQTYDDLLAKDCHCI

SEQ ID NO: 39 - protein, 109 aa, synthetic construct
GDHCPLGPGRCCRLHTVRASLEDLGWADWVLSPREVQVTMCIGACPSQFRAANMHAQIKTSLHRLKPDTVPAPCCVPASYNPMVLIQKTDTGVSLQTYDDLLAKDCHCI

SEQ ID NO: 40 - protein, 108 aa, synthetic construct
DHCPLGPGRCCRLHTVRASLEDLGWADWVLSPREVQVTMCIGACPSQFRAANMHAQIKTSLHRLKPDTVPAPCCVPASYNPMVLIQKTDTGVSLQTYDDLLAKDCHCI

SEQ ID NO: 41 - protein, 98 aa, synthetic construct
CRLHTVRASLEDLGWADWVLSPREVQVTMCIGACPSQFRAANMHAQIKTSLHRLKPDTVPAPCCVPASYNPMVLIQKTDTGVSLQTYDDLLAKDCHCI

SEQ ID NO: 42 - protein, 108 aa, synthetic construct
EHCPLGPGRCCRLHTVRASLEDLGWADWVLSPREVQVTMCIGACPSQFRAANMHAQIKTSLHRLKPDTVPAPCCVPASYNPMVLIQKTDTGVSLQTYDDLLAKDCHCI

SEQ ID NO: 43 - protein, 107 aa, synthetic construct
DCPLGPGRCCRLHTVRASLEDLGWADWVLSPREVQVTMCIGACPSQFRAANMHAQIKTSLHRLKPDTVPAPCCVPASYNPMVLIQKTDTGVSLQTYDDLLAKDCHCI

SEQ ID NO: 44 - protein, 108 aa, synthetic construct
DECPLGPGRCCRLHTVRASLEDLGWADWVLSPREVQVTMCIGACPSQFRAANMHAQIKTSLHRLKPDTVPAPCCVPASYNPMVLIQKTDTGVSLQTYDDLLAKDCHCI

SEQ ID NO: 45 - protein, 107 aa, synthetic construct
ECPLGPGRCCRLHTVRASLEDLGWADWVLSPREVQVTMCIGACPSQFRAANMHAQIKTSLHRLKPDTVPAPCCVPASYNPMVLIQKTDTGVSLQTYDDLLAKDCHCI

SEQ ID NO: 46 - protein, 108 aa, synthetic construct
DHCPLGPGRCCRLHTVQASLEDLGWADWVLSPREVQVTMCIGACPSQFRAANMHAQIKTSLHRLKPDTVPAPCCVPASYNPMVLIQKTDTGVSLQTYDDLLAKDCHCI

SEQ ID NO: 47 - protein, 108 aa, synthetic construct
DHCPLGPGRCCRLHTVHASLEDLGWADWVLSPREVQVTMCIGACPSQFRAANMHAQIKTSLHRLKPDTVPAPCCVPASYNPMVLIQKTDTGVSLQTYDDLLAKDCHCI

SEQ ID NO: 48 - protein, 108 aa, synthetic construct
DHCPLGPGRCCRLHTVRASLEELGWADWVLSPREVQVTMCIGACPSQFRAANMHAQIKTSLHRLKPDTVPAPCCVPASYNPMVLIQKTDTGVSLQTYDDLLAKDCHCI

SEQ ID NO: 49 - protein, 108 aa, synthetic construct
DHCPLGPGRCCRLHTVRASLEELGWADWVLSPREVQVTMCIGACPSQFRAANMHAQIKTSLHRLRPDTVPAPCCVPASYNPMVLIQKTDTGVSLQTYDDLLAKDCHCI

SEQ ID NO: 50 - protein, 108 aa, synthetic construct
DHCPLGPGRCCRLHTVRASLEDLGWSDWVLSPREVQVTMCIGACPSQFRAANMHAQIKTSLHRLKPDTVPAPCCVPASYNPMVLIQKTDTGVSLQTYDDLLAKDCHCI

SEQ ID NO: 51 - protein, 108 aa, synthetic construct
DHCPLGPGRCCRLHTVRASLEDLGWADWVLSPREVQVTMCIGDCPSQFRAANMHAQIKTSLHRLKPDTVPAPCCVPASYNPMVLIQKTDTGVSLQTYDDLLAKDCHCI

SEQ ID NO: 52 - protein, 108 aa, synthetic construct
DHCPLGPGRCCRLHTVRASLEDLGWADWVLSPREVQVTMCIGACPSQFRSANMHAQIKTSLHRLKPDTVPAPCCVPASYNPMVLIQKTDTGVSLQTYDDLLAKDCHCI

SEQ ID NO: 53 - protein, 108 aa, synthetic construct
DHCPLGPGRCCRLHTVRASLEDLGWADWVLSPREVQVTMCIGACPSQFRAENMHAQIKTSLHRLKPDTVPAPCCVPASYNPMVLIQKTDTGVSLQTYDDLLAKDCHCI

SEQ ID NO: 54 - protein, 108 aa, synthetic construct
DHCPLGPGRCCRLHTVRASLEDLGWADWVLSPREVQVTMCIGACPSQFRAANTHAQIKTSLHRLKPDTVPAPCCVPASYNPMVLIQKTDTGVSLQTYDDLLAKDCHCI

SEQ ID NO: 55 - protein, 108 aa, synthetic construct
DHCPLGPGRCCRLHTVRASLEDLGWADWVLSPREVQVTMCIGACPSQFRAANMHAQIKTSLHQLKPDTVPAPCCVPASYNPMVLIQKTDTGVSLQTYDDLLAKDCHCI

SEQ ID NO: 56 - protein, 108 aa, synthetic construct
DHCPLGPGRCCRLHTVRASLEDLGWADWVLSPREVQVTMCIGACPSQFRAANMHAQIKTSLHRLKPDTVPAPCCVPSSYNPMVLIQKTDTGVSLQTYDDLLAKDCHCI

SEQ ID NO: 57 - protein, 108 aa, synthetic construct
DHCPLGPGRCCRLHTVRASLEDLGWADWVLSPREVQVTMCIGACPSQFRAANMHAQIKTSLHRLKPDTVPAPCCVPASYNPMVLIQKTDEGVSLQTYDDLLAKDCHCI

SEQ ID NO: 58 - protein, 108 aa, synthetic construct
DHCPLGPGRCCRLHTVRASLEDLGWADWVLSPREVQVTMCIGACPSQFRAANMHAQIKTSLHRLKPDTVPAPCCVPASYNPMVLIQKTDTGVSLQTYDDLLAQDCHCI

SEQ ID NO: 59 - protein, 414 aa, synthetic construct
HAEGTFTSDVSSYLEGQAAKEFIAWLVKGRGGGGGSGGGGSGGGGSAPEAAGGPSVFLFPPKPKDTLMISRTPEVTCVVVDVSQEDPEVQFNWYVDGVEVHNAKTKPREEQFNSTYRVVSVLTVLHQDWLNGKEYKCKVSNKGLPSSIEKTISKAKGQPREPQVYTLPPSQEEMTKNQVSLTCLVKGFYPSDIAVEWESNGQPENNYKTTPPVLDSDGSFFLYSRLTVDKSRWQEGNVFSCSVMHEALHNHYTQKSLSLSLGGGGGSGGGGSAPAPAPAPAPAPAPAPAPAPGGGGSGGGGSARNGDHCPLGPGRCCRLHTVRASLEDLGWADWVLSPREVQVTMCIGACPSQFRAANMHAQIKTSLHRLKPDTVPAPCCVPASYNPMVLIQKTDTGVSLQTYDDLLAKDCHCI

SEQ ID NO: 60 - protein, 414 aa, synthetic construct
HAEGTFTSDVSSYLEGQAAKEFIAWLVKGRGGGGGSGGGGSGGGGSAPEAAGGPSVFLFPPKPKDTLMISRTPEVTCVVVDVSQEDPEVQFNWYVDGVEVHNAKTKPREEQFNSTYRVVSVLTVLHQDWLNGKEYKCKVSNKGLPSSIEKTISKAKGQPREPQVYTLPPSQEEMTKNQVSLTCLVKGFYPSDIAVEWESNGQPENNYKTTPPVLDSDGSFFLYSRLTVDKSRWQEGNVFSCSVMHEALHNHYTQESLSLSLGGGGGSGGGGSAPAPAPAPAPAPAPAPAPAPGGGGSGGGGSARNGDHCPLGPGRCCRLHTVRASLEDLGWADWVLSPREVQVTMCIGACPSQFRAANMHAQIKTSLHRLKPDTVPAPCCVPASYNPMVLIQKTDTGVSLQTYDDLLAKDCHCI

SEQ ID NO: 61 - protein, 414 aa, synthetic construct
HAEGTFTSDVSSYLEGQAAKEFIAWLVKGRGGGGGSGGGGSGGGGSAPEAAGGPSVFLFPPKPKDTLMISRTPEVTCVVVDVSQEDPEVQFNWYVDGVEVHNAKTKPREEQFNSTYRVVSVLTVLHQDWLNGKEYKCKVSNKGLPSSIEKTISKAKGQPREPQVYTLPPSQEEMTKNQVSLTCLVKGFYPSDIAVEWESNGQPENNYKTTPPVLDSDGSFFLYSRLTVDKSRWQEGNVFSCSVMHEALHNHYTQQSLSLSLGGGGGSGGGGSAPAPAPAPAPAPAPAPAPAPGGGGSGGGGSARNGDHCPLGPGRCCRLHTVRASLEDLGWADWVLSPREVQVTMCIGACPSQFRAANMHAQIKTSLHRLKPDTVPAPCCVPASYNPMVLIQKTDTGVSLQTYDDLLAKDCHCI

SEQ ID NO: 62 - protein, 412 aa, synthetic construct
HAEGTFTSDVSSYLEGQAAKEFIAWLVKGRGGGGGSGGGGSGGGGSEAAGGPSVFLFPPKPKDTLMISRTPEVTCVVVDVSQEDPEVQFNWYVDGVEVHNAKTKPREEQFNSTYRVVSVLTVLHQDWLNGKEYKCKVSNKGLPSSIEKTISKAKGQPREPQVYTLPPSQEEMTKNQVSLTCLVKGFYPSDIAVEWESNGQPENNYKTTPPVLDSDGSFFLYSRLTVDKSRWQEGNVFSCSVMHEALHNHYTQKSLSLSLGGGGGSGGGGSAPAPAPAPAPAPAPAPAPAPGGGGSGGGGSARNGDHCPLGPGRCCRLHTVRASLEDLGWADWVLSPREVQVTMCIGACPSQFRAANMHAQIKTSLHRLKPDTVPAPCCVPASYNPMVLIQKTDTGVSLQTYDDLLAKDCHCI

SEQ ID NO: 63 - protein, 412 aa, synthetic construct
HAEGTFTSDVSSYLEGQAAKEFIAWLVKGRGGGGGSGGGGSGGGGSEAAGGPSVFLFPPKPKDTLMISRTPEVTCVVVDVSQEDPEVQFNWYVDGVEVHNAKTKPREEQFNSTYRVVSVLTVLHQDWLNGKEYKCKVSNKGLPSSIEKTISKAKGQPREPQVYTLPPSQEEMTKNQVSLTCLVKGFYPSDIAVEWESNGQPENNYKTTPPVLDSDGSFFLYSRLTVDKSRWQEGNVFSCSVMHEALHNHYTQESLSLSLGGGGGSGGGGSAPAPAPAPAPAPAPAPAPAPGGGGSGGGGSARNGDHCPLGPGRCCRLHTVRASLEDLGWADWVLSPREVQVTMCIGACPSQFRAANMHAQIKTSLHRLKPDTVPAPCCVPASYNPMVLIQKTDTGVSLQTYDDLLAKDCHCI

SEQ ID NO: 64 - protein, 412 aa, synthetic construct
HAEGTFTSDVSSYLEGQAAKEFIAWLVKGRGGGGGSGGGGSGGGGSEAAGGPSVFLFPPKPKDTLMISRTPEVTCVVVDVSQEDPEVQFNWYVDGVEVHNAKTKPREEQFNSTYRVVSVLTVLHQDWLNGKEYKCKVSNKGLPSSIEKTISKAKGQPREPQVYTLPPSQEEMTKNQVSLTCLVKGFYPSDIAVEWESNGQPENNYKTTPPVLDSDGSFFLYSRLTVDKSRWQEGNVFSCSVMHEALHNHYTQQSLSLSLGGGGGSGGGGSAPAPAPAPAPAPAPAPAPAPGGGGSGGGGSARNGDHCPLGPGRCCRLHTVRASLEDLGWADWVLSPREVQVTMCIGACPSQFRAANMHAQIKTSLHRLKPDTVPAPCCVPASYNPMVLIQKTDTGVSLQTYDDLLAKDCHCI

SEQ ID NO: 65 - protein, 410 aa, synthetic construct
HGEGTFTSDVSSYLEEQAAKEFIAWLVKGGGGGGGSGGGGSGGGGSAPEAAGGPSVFLFPPKPKDTLMISRTPEVTCVVVDVSQEDPEVQFNWYVDGVEVHNAKTKPREEQFNSTYRVVSVLTVLHQDWLNGKEYKCKVSNKGLPSSIEKTISKAKGQPREPQVYTLPPSQEEMTKNQVSLTCLVKGFYPSDIAVEWESNGQPENNYKTTPPVLDSDGSFFLYSRLTVDKSRWQEGNVFSCSVMHEALHNHYTQKSLSLSLGGGGGSGGGGSAPAPAPAPAPAPAPAPAPAPGGGGSGGGGSDHCPLGPGRCCRLHTVRASLEDLGWADWVLSPREVQVTMCIGACPSQFRAANMHAQIKTSLHRLKPDTVPAPCCVPASYNPMVLIQKTDTGVSLQTYDDLLAKDCHCI

SEQ ID NO: 66 - protein, 410 aa, synthetic construct
HGEGTFTSDVSSYLEEQAAKEFIAWLVKGGGGGGGSGGGGSGGGGSAPEAAGGPSVFLFPPKPKDTLMISRTPEVTCVVVDVSQEDPEVQFNWYVDGVEVHNAKTKPREEQFNSTYRVVSVLTVLHQDWLNGKEYKCKVSNKGLPSSIEKTISKAKGQPREPQVYTLPPSQEEMTKNQVSLTCLVKGFYPSDIAVEWESNGQPENNYKTTPPVLDSDGSFFLYSRLTVDKSRWQEGNVFSCSVMHEALHNHYTQESLSLSLGGGGGSGGGGSAPAPAPAPAPAPAPAPAPAPGGGGSGGGGSDHCPLGPGRCCRLHTVRASLEDLGWADWVLSPREVQVTMCIGACPSQFRAANMHAQIKTSLHRLKPDTVPAPCCVPASYNPMVLIQKTDTGVSLQTYDDLLAKDCHCI

SEQ ID NO: 67 - protein, 410 aa, synthetic construct
HGEGTFTSDVSSYLEEQAAKEFIAWLVKGGGGGGGSGGGGSGGGGSAPEAAGGPSVFLFPPKPKDTLMISRTPEVTCVVVDVSQEDPEVQFNWYVDGVEVHNAKTKPREEQFNSTYRVVSVLTVLHQDWLNGKEYKCKVSNKGLPSSIEKTISKAKGQPREPQVYTLPPSQEEMTKNQVSLTCLVKGFYPSDIAVEWESNGQPENNYKTTPPVLDSDGSFFLYSRLTVDKSRWQEGNVFSCSVMHEALHNHYTQQSLSLSLGGGGGSGGGGSAPAPAPAPAPAPAPAPAPAPGGGGSGGGGSDHCPLGPGRCCRLHTVRASLEDLGWADWVLSPREVQVTMCIGACPSQFRAANMHAQIKTSLHRLKPDTVPAPCCVPASYNPMVLIQKTDTGVSLQTYDDLLAKDCHCI

SEQ ID NO: 68 - protein, 408 aa, synthetic construct
HGEGTFTSDVSSYLEEQAAKEFIAWLVKGGGGGGGSGGGGSGGGGSEAAGGPSVFLFPPKPKDTLMISRTPEVTCVVVDVSQEDPEVQFNWYVDGVEVHNAKTKPREEQFNSTYRVVSVLTVLHQDWLNGKEYKCKVSNKGLPSSIEKTISKAKGQPREPQVYTLPPSQEEMTKNQVSLTCLVKGFYPSDIAVEWESNGQPENNYKTTPPVLDSDGSFFLYSRLTVDKSRWQEGNVFSCSVMHEALHNHYTQKSLSLSLGGGGGSGGGGSAPAPAPAPAPAPAPAPAPAPGGGGSGGGGSDHCPLGPGRCCRLHTVRASLEDLGWADWVLSPREVQVTMCIGACPSQFRAANMHAQIKTSLHRLKPDTVPAPCCVPASYNPMVLIQKTDTGVSLQTYDDLLAKDCHCI

SEQ ID NO: 69 - protein, 408 aa, synthetic construct
HGEGTFTSDVSSYLEEQAAKEFIAWLVKGGGGGGGSGGGGSGGGGSEAAGGPSVFLFPPKPKDTLMISRTPEVTCVVVDVSQEDPEVQFNWYVDGVEVHNAKTKPREEQFNSTYRVVSVLTVLHQDWLNGKEYKCKVSNKGLPSSIEKTISKAKGQPREPQVYTLPPSQEEMTKNQVSLTCLVKGFYPSDIAVEWESNGQPENNYKTTPPVLDSDGSFFLYSRLTVDKSRWQEGNVFSCSVMHEALHNHYTQESLSLSLGGGGGSGGGGSAPAPAPAPAPAPAPAPAPAPGGGGSGGGGSDHCPLGPGRCCRLHTVRASLEDLGWADWVLSPREVQVTMCIGACPSQFRAANMHAQIKTSLHRLKPDTVPAPCCVPASYNPMVLIQKTDTGVSLQTYDDLLAKDCHCI

SEQ ID NO: 70 - protein, 408 aa, synthetic construct
HGEGTFTSDVSSYLEEQAAKEFIAWLVKGGGGGGGSGGGGSGGGGSEAAGGPSVFLFPPKPKDTLMISRTPEVTCVVVDVSQEDPEVQFNWYVDGVEVHNAKTKPREEQFNSTYRVVSVLTVLHQDWLNGKEYKCKVSNKGLPSSIEKTISKAKGQPREPQVYTLPPSQEEMTKNQVSLTCLVKGFYPSDIAVEWESNGQPENNYKTTPPVLDSDGSFFLYSRLTVDKSRWQEGNVFSCSVMHEALHNHYTQQSLSLSLGGGGGSGGGGSAPAPAPAPAPAPAPAPAPAPGGGGSGGGGSDHCPLGPGRCCRLHTVRASLEDLGWADWVLSPREVQVTMCIGACPSQFRAANMHAQIKTSLHRLKPDTVPAPCCVPASYNPMVLIQKTDTGVSLQTYDDLLAKDCHCI

SEQ ID NO: 71 - protein, 408 aa, synthetic construct
HGEGTFTSDVSSYLEEQAAKEFIQWLVKGGGGGGGSGGGGSGGGGSEAAGGPSVFLFPPKPKDTLMISRTPEVTCVVVDVSQEDPEVQFNWYVDGVEVHNAKTKPREEQFNSTYRVVSVLTVLHQDWLNGKEYKCKVSNKGLPSSIEKTISKAKGQPREPQVYTLPPSQEEMTKNQVSLTCLVKGFYPSDIAVEWESNGQPENNYKTTPPVLDSDGSFFLYSRLTVDKSRWQEGNVFSCSVMHEALHNHYTQESLSLSLGGGGGSGGGGSAPAPAPAPAPAPAPAPAPAPGGGGSGGGGSDHCPLGPGRCCRLHTVRASLEDLGWADWVLSPREVQVTMCIGACPSQFRAANMHAQIKTSLHRLKPDTVPAPCCVPASYNPMVLIQKTDTGVSLQTYDDLLAKDCHCI

SEQ ID NO: 72 - protein, 408 aa, synthetic construct
HGEGTFTSDVSSYLEEQAAKEFVQWLVKGGGGGGGSGGGGSGGGGSEAAGGPSVFLFPPKPKDTLMISRTPEVTCVVVDVSQEDPEVQFNWYVDGVEVHNAKTKPREEQFNSTYRVVSVLTVLHQDWLNGKEYKCKVSNKGLPSSIEKTISKAKGQPREPQVYTLPPSQEEMTKNQVSLTCLVKGFYPSDIAVEWESNGQPENNYKTTPPVLDSDGSFFLYSRLTVDKSRWQEGNVFSCSVMHEALHNHYTQESLSLSLGGGGGSGGGGSAPAPAPAPAPAPAPAPAPAPGGGGSGGGGSDHCPLGPGRCCRLHTVRASLEDLGWADWVLSPREVQVTMCIGACPSQFRAANMHAQIKTSLHRLKPDTVPAPCCVPASYNPMVLIQKTDTGVSLQTYDDLLAKDCHCI

SEQ ID NO: 73 - protein, 423 aa, synthetic construct
HGEGTFTSDVSSYLEEQAAKEFIAWLVKGGGGGGGSGGGGSGGGGSAESKYGPPCPPCPAPEAAGGPSVFLFPPKPKDTLMISRTPEVTCVVVDVSQEDPEVQFNWYVDGVEVHNAKTKPREEQFNSTYRVVSVLTVLHQDWLNGKEYKCKVSNKGLPSSIEKTISKAKGQPREPQVYTLPPSQEEMTKNQVSLTCLVKGFYPSDIAVEWESNGQPENNYKTTPPVLDSDGSFFLYSRLTVDKSRWQEGNVFSCSVMHEALHNHYTQESLSLSLGGGGGSGGGGSAPAPAPAPAPAPAPAPAPAPGGGGSGGGGSDHCPLGPGRCCRLHTVRASLEDLGWADWVLSPREVQVTMCIGACPSQFRAANMHAQIKTSLHRLKPDTVPAPCCVPASYNPMVLIQKTDTGVSLQTYDDLLAKDCHCI

SEQ ID NO: 74 - protein, 410 aa, synthetic construct
HGEGTFTSDVSSYLEEQAAKEFIAWLVKGGGGGGGSGGGGSGGGGSAPEAAGGPSVFLFPPKPKDTLMISRTPEVTCVVVDVSHEDPEVKFNWYVDGVEVHNAKTKPREEQYNSTYRVVSVLTVLHQDWLNGKEYKCKVSNKALPAPIEKTISKAKGQPREPQVYTLPPSRDELTKNQVSLTCLVKGFYPSDIAVEWESNGQPENNYKTTPPVLDSDGSFFLYSKLTVDKSRWQQGNVFSCSVMHEALHNHYTQESLSLSPGGGGGSGGGGSAPAPAPAPAPAPAPAPAPAPGGGGSGGGGSDHCPLGPGRCCRLHTVRASLEDLGWADWVLSPREVQVTMCIGACPSQFRAANMHAQIKTSLHRLKPDTVPAPCCVPASYNPMVLIQKTDTGVSLQTYDDLLAKDCHCI

SEQ ID NO: 75 - protein, 410 aa, synthetic construct
HGEGTFTSDVSSYLEEQAAKEFIQWLVKGGGGGGGSGGGGSGGGGSAPEAAGGPSVFLFPPKPKDTLMISRTPEVTCVVVDVSHEDPEVKFNWYVDGVEVHNAKTKPREEQYNSTYRVVSVLTVLHQDWLNGKEYKCKVSNKALPAPIEKTISKAKGQPREPQVYTLPPSRDELTKNQVSLTCLVKGFYPSDIAVEWESNGQPENNYKTTPPVLDSDGSFFLYSKLTVDKSRWQQGNVFSCSVMHEALHNHYTQESLSLSPGGGGGSGGGGSAPAPAPAPAPAPAPAPAPAPGGGGSGGGGSDHCPLGPGRCCRLHTVRASLEDLGWADWVLSPREVQVTMCIGACPSQFRAANMHAQIKTSLHRLKPDTVPAPCCVPASYNPMVLIQKTDTGVSLQTYDDLLAKDCHCI

SEQ ID NO: 76 - protein, 410 aa, synthetic construct
HGEGTFTSDVSSYLEEQAAKEFVQWLVKGGGGGGGSGGGGSGGGGSAPEAAGGPSVFLFPPKPKDTLMISRTPEVTCVVVDVSHEDPEVKFNWYVDGVEVHNAKTKPREEQYNSTYRVVSVLTVLHQDWLNGKEYKCKVSNKALPAPIEKTISKAKGQPREPQVYTLPPSRDELTKNQVSLTCLVKGFYPSDIAVEWESNGQPENNYKTTPPVLDSDGSFFLYSKLTVDKSRWQQGNVFSCSVMHEALHNHYTQESLSLSPGGGGGSGGGGSAPAPAPAPAPAPAPAPAPAPGGGGSGGGGSDHCPLGPGRCCRLHTVRASLEDLGWADWVLSPREVQVTMCIGACPSQFRAANMHAQIKTSLHRLKPDTVPAPCCVPASYNPMVLIQKTDTGVSLQTYDDLLAKDCHCI

SEQ ID NO: 77 - protein, 420 aa, synthetic construct
HGEGTFTSDVSSYLEEQAAKEFIAWLVKGGGGGGGSGGGGSGGGGSDKTHTCPPCPAPEAAGGPSVFLFPPKPKDTLMISRTPEVTCVVVDVSHEDPEVKFNWYVDGVEVHNAKTKPREEQYNSTYRVVSVLTVLHQDWLNGKEYKCKVSNKALPAPIEKTISKAKGQPREPQVYTLPPSRDELTKNQVSLTCLVKGFYPSDIAVEWESNGQPENNYKTTPPVLDSDGSFFLYSKLTVDKSRWQQGNVFSCSVMHEALHNHYTQESLSLSPGGGGGSGGGGSAPAPAPAPAPAPAPAPAPAPGGGGSGGGGSDHCPLGPGRCCRLHTVRASLEDLGWADWVLSPREVQVTMCIGACPSQFRAANMHAQIKTSLHRLKPDTVPAPCCVPASYNPMVLIQKTDTGVSLQTYDDLLAKDCHCI

SEQ ID NO: 78 - protein, 15 aa, synthetic construct
GGGGSGGGGSGGGGS

SEQ ID NO: 79 - protein, 28 aa, synthetic construct
GGGGAPAPAPAPAPAPAPAPAPAPGGGG

SEQ ID NO: 80 - protein, 40 aa, synthetic construct
GGGGSGGGGSAPAPAPAPAPAPAPAPAPAPGGGGSGGGGS

SEQ ID NO: 81 - protein, 40 aa, synthetic construct
GGGGSGGGGSEPEPEPEPEPEPEPEPEPEPGGGGSGGGGS

SEQ ID NO: 82 - protein, 214 aa, synthetic construct
EAAGGPSVFLFPPKPKDTLMISRTPEVTCVVVDVSQEDPEVQFNWYVDGVEVHNAKTKPREEQFNSTYRVVSVLTVLHQDWLNGKEYKCKVSNKGLPSSIEKTISKAKGQPREPQVYTLPPSQEEMTKNQVSLTCLVKGFYPSDIAVEWESNGQPENNYKTTPPVLDSDGSFQLESRLTVDKSRWQEGNVFSCSVMHEALHNHYTQKSLSLSLG

SEQ ID NO: 83 - protein, 364 aa, synthetic construct
APEAAGGPSVFLFPPKPKDTLMISRTPEVTCVVVDVSQEDPEVQFNWYVDGVEVHNAKTKPREEQFNSTYRVVSVLTVLHQDWLNGKEYKCKVSNKGLPSSIEKTISKAKGQPREPQVYTLPPSQEEMTKNQVSLTCLVKGFYPSDIAVEWESNGQPENNYKTTPPVLDSDGSFFLYSRLTVDKSRWQEGNVFSCSVMHEALHNHYTQKSLSLSLGGGGGSGGGGSAPAPAPAPAPAPAPAPAPAPGGGGSGGGGSDHCPLGPGRCCRLHTVRASLEDLGWADWVLSPREVQVTMCIGACPSQFRAANMHAQIKTSLHRLKPDTVPAPCCVPASYNPMVLIQKTDTGVSLQTYDDLLAKDCHCI

SEQ ID NO: 84 - protein, 368 aa, synthetic construct
APEAAGGPSVFLFPPKPKDTLMISRTPEVTCVVVDVSQEDPEVQFNWYVDGVEVHNAKTKPREEQFNSTYRVVSVLTVLHQDWLNGKEYKCKVSNKGLPSSIEKTISKAKGQPREPQVYTLPPSQEEMTKNQVSLTCLVKGFYPSDIAVEWESNGQPENNYKTTPPVLDSDGSFFLYSRLTVDKSRWQEGNVFSCSVMHEALHNHYTQESLSLSLGGGGGSGGGGSAPAPAPAPAPAPAPAPAPAPGGGGSGGGGSARNGDHCPLGPGRCCRLHTVRASLEDLGWADWVLSPREVQVTMCIGACPSQFRAANMHAQIKTSLHRLKPDTVPAPCCVPASYNPMVLIQKTDTGVSLQTYDDLLAKDCHCI

SEQ ID NO: 85 - protein, 365 aa, synthetic construct
APEAAGGPSVFLFPPKPKDTLMISRTPEVTCVVVDVSQEDPEVQFNWYVDGVEVHNAKTKPREEQFNSTYRVVSVLTVLHQDWLNGKEYKCKVSNKGLPSSIEKTISKAKGQPREPQVYTLPPSQEEMTKNQVSLTCLVKGFYPSDIAVEWESNGQPENNYKTTPPVLDSDGSFFLYSRLTVDKSRWQEGNVFSCSVMHEALHNHYTQESLSLSLGGGGGSGGGGSAPAPAPAPAPAPAPAPAPAPGGGGSGGGGSGDHCPLGPGRCCRLHTVRASLEDLGWADWVLSPREVQVTMCIGACPSQFRAANMHAQIKTSLHRLKPDTVPAPCCVPASYNPMVLIQKTDTGVSLQTYDDLLAKDCHCI

SEQ ID NO: 86 - protein, 364 aa, synthetic construct
APEAAGGPSVFLFPPKPKDTLMISRTPEVTCVVVDVSQEDPEVQFNWYVDGVEVHNAKTKPREEQFNSTYRVVSVLTVLHQDWLNGKEYKCKVSNKGLPSSIEKTISKAKGQPREPQVYTLPPSQEEMTKNQVSLTCLVKGFYPSDIAVEWESNGQPENNYKTTPPVLDSDGSFFLYSRLTVDKSRWQEGNVFSCSVMHEALHNHYTQESLSLSLGGGGGSGGGGSAPAPAPAPAPAPAPAPAPAPGGGGSGGGGSDHCPLGPGRCCRLHTVRASLEDLGWADWVLSPREVQVTMCIGACPSQFRAANMHAQIKTSLHRLKPDTVPAPCCVPASYNPMVLIQKTDTGVSLQTYDDLLAKDCHCI

SEQ ID NO: 87 - protein, 364 aa, synthetic construct
APEAAGGPSVFLFPPKPKDTLMISRTPEVTCVVVDVSQEDPEVQFNWYVDGVEVHNAKTKPREEQFNSTYRVVSVLTVLHQDWLNGKEYKCKVSNKGLPSSIEKTISKAKGQPREPQVYTLPPSQEEMTKNQVSLTCLVKGFYPSDIAVEWESNGQPENNYKTTPPVLDSDGSFFLYSRLTVDKSRWQEGNVFSCSVMHEALHNHYTQDSLSLSLGGGGGSGGGGSAPAPAPAPAPAPAPAPAPAPGGGGSGGGGSDHCPLGPGRCCRLHTVRASLEDLGWADWVLSPREVQVTMCIGACPSQFRAANMHAQIKTSLHRLKPDTVPAPCCVPASYNPMVLIQKTDTGVSLQTYDDLLAKDCHCI

SEQ ID NO: 88 - protein, 364 aa, synthetic construct
APEAAGGPSVFLFPPKPKDTLMISRTPEVTCVVVDVSQEDPEVQFNWYVDGVEVHNAKTKPREEQFNSTYRVVSVLTVLHQDWLNGKEYKCKVSNKGLPSSIEKTISKAKGQPREPQVYTLPPSQEEMTKNQVSLTCLVKGFYPSDIAVEWESNGQPENNYKTTPPVLDSDGSFFLYSRLTVDKSRWQEGNVFSCSVMHEALHNHYTQQSLSLSLGGGGGSGGGGSAPAPAPAPAPAPAPAPAPAPGGGGSGGGGSDHCPLGPGRCCRLHTVRASLEDLGWADWVLSPREVQVTMCIGACPSQFRAANMHAQIKTSLHRLKPDTVPAPCCVPASYNPMVLIQKTDTGVSLQTYDDLLAKDCHCI

SEQ ID NO: 89 - protein, 364 aa, synthetic construct
APEAAGGPSVFLFPPKPKDTLMISRTPEVTCVVVDVSQEDPEVQFNWYVDGVEVHNAKTKPREEQFNSTYRVVSVLTVLHQDWLNGKEYKCKVSNKGLPSSIEKTISKAKGQPREPQVYTLPPSQEEMTKNQVSLTCLVKGFYPSDIAVEWESNGQPENNYKTTPPVLDSDGSFFLYSRLTVDKSRWQEGNVFSCSVMHEALHNHYTQASLSLSLGGGGGSGGGGSAPAPAPAPAPAPAPAPAPAPGGGGSGGGGSDHCPLGPGRCCRLHTVRASLEDLGWADWVLSPREVQVTMCIGACPSQFRAANMHAQIKTSLHRLKPDTVPAPCCVPASYNPMVLIQKTDTGVSLQTYDDLLAKDCHCI

SEQ ID NO: 90 - protein, 364 aa, synthetic construct
APEAAGGPSVFLFPPKPKDTLMISRTPEVTCVVVDVSQEDPEVQFNWYVDGVEVHNAKTKPREEQFNSTYRVVSVLTVLHQDWLNGKEYKCKVSNKGLPSSIEKTISKAKGQPREPQVYTLPPSQKEMTKNQVSLTCLVKGFYPSDIAVEWESNGQPENNYKTTPPVLDSDGSFFLYSRLTVDKSRWQEGNVFSCSVMHEALHNHYTQKSLSLSLGGGGGSGGGGSAPAPAPAPAPAPAPAPAPAPGGGGSGGGGSDHCPLGPGRCCRLHTVRASLEDLGWADWVLSPREVQVTMCIGACPSQFRAANMHAQIKTSLHRLKPDTVPAPCCVPASYNPMVLIQKTDTGVSLQTYDDLLAKDCHCI

SEQ ID NO: 91 - protein, 364 aa, synthetic construct
APEAAGGPSVFLFPPKPKDTLMISRTPEVTCVVVDVSQEDPEVQFNWYVDGVEVHNAKTKPREEQFNSTYRVVSVLTVLHQDWLNGKEYKCKVSNKGLPSSIEKTISKAKGQPREPQVYTLPPSQREMTKNQVSLTCLVKGFYPSDIAVEWESNGQPENNYKTTPPVLDSDGSFFLYSRLTVDKSRWQEGNVFSCSVMHEALHNHYTQKSLSLSLGGGGGSGGGGSAPAPAPAPAPAPAPAPAPAPGGGGSGGGGSDHCPLGPGRCCRLHTVRASLEDLGWADWVLSPREVQVTMCIGACPSQFRAANMHAQIKTSLHRLKPDTVPAPCCVPASYNPMVLIQKTDTGVSLQTYDDLLAKDCHCI

SEQ ID NO: 92 - protein, 364 aa, synthetic construct
APEAAGGPSVFLFPPKPKDTLMISRTPEVTCVVVDVSQEDPEVQFNWYVDGVEVHNAKTKPREEQFNSTYRVVSVLTVLHQDWLNGKEYKCKVSNKGLPSSIEKTISKAKGQPREPQVYTLPPSQQEMTKNQVSLTCLVKGFYPSDIAVEWESNGQPENNYKTTPPVLDSDGSFFLYSRLTVDKSRWQEGNVFSCSVMHEALHNHYTQKSLSLSLGGGGGSGGGGSAPAPAPAPAPAPAPAPAPAPGGGGSGGGGSDHCPLGPGRCCRLHTVRASLEDLGWADWVLSPREVQVTMCIGACPSQFRAANMHAQIKTSLHRLKPDTVPAPCCVPASYNPMVLIQKTDTGVSLQTYDDLLAKDCHCI

SEQ ID NO: 93 - protein, 364 aa, synthetic construct
APEAAGGPSVFLFPPKPKDTLMISRTPEVTCVVVDVSQEDPEVQFNWYVDGVEVHNAKTKPREEQFNSTYRVVSVLTVLHQDWLNGKEYKCKVSNKGLPSSIEKTISKAKGQPREPQVYTLPPSQAEMTKNQVSLTCLVKGFYPSDIAVEWESNGQPENNYKTTPPVLDSDGSFFLYSRLTVDKSRWQEGNVFSCSVMHEALHNHYTQKSLSLSLGGGGGSGGGGSAPAPAPAPAPAPAPAPAPAPGGGGSGGGGSDHCPLGPGRCCRLHTVRASLEDLGWADWVLSPREVQVTMCIGACPSQFRAANMHAQIKTSLHRLKPDTVPAPCCVPASYNPMVLIQKTDTGVSLQTYDDLLAKDCHCI

SEQ ID NO: 94 - protein, 364 aa, synthetic construct
APEAAGGPSVFLFPPKPKDTLMISRTPEVTCVVVDVSHEDPEVKFNWYVDGVEVHNAKTKPREEQYNSTYRVVSVLTVLHQDWLNGKEYKCKVSNKALPAPIEKTISKAKGQPREPQVYTLPPSRDELTKNQVSLTCLVKGFYPSDIAVEWESNGQPENNYKTTPPVLDSDGSFFLYSKLTVDKSRWQQGNVFSCSVMHEALHNHYTQESLSLSPGGGGGSGGGGSAPAPAPAPAPAPAPAPAPAPGGGGSGGGGSDHCPLGPGRCCRLHTVRASLEDLGWADWVLSPREVQVTMCIGACPSQFRAANMHAQIKTSLHRLKPDTVPAPCCVPASYNPMVLIQKTDTGVSLQTYDDLLAKDCHCI

SEQ ID NO: 95 - protein, 362 aa, synthetic construct
EAAGGPSVFLFPPKPKDTLMISRTPEVTCVVVDVSQEDPEVQFNWYVDGVEVHNAKTKPREEQFNSTYRVVSVLTVLHQDWLNGKEYKCKVSNKGLPSSIEKTISKAKGQPREPQVYTLPPSQEEMTKNQVSLTCLVKGFYPSDIAVEWESNGQPENNYKTTPPVLDSDGSFFLYSRLTVDKSRWQEGNVFSCSVMHEALHNHYTQESLSLSLGGGGGSGGGGSAPAPAPAPAPAPAPAPAPAPGGGGSGGGGSDHCPLGPGRCCRLHTVRASLEDLGWADWVLSPREVQVTMCIGACPSQFRAANMHAQIKTSLHRLKPDTVPAPCCVPASYNPMVLIQKTDTGVSLQTYDDLLAKDCHCI

SEQ ID NO: 96 - protein, 359 aa, synthetic construct
GGPSVFLFPPKPKDTLMISRTPEVTCVVVDVSQEDPEVQFNWYVDGVEVHNAKTKPREEQFNSTYRVVSVLTVLHQDWLNGKEYKCKVSNKGLPSSIEKTISKAKGQPREPQVYTLPPSQEEMTKNQVSLTCLVKGFYPSDIAVEWESNGQPENNYKTTPPVLDSDGSFFLYSRLTVDKSRWQEGNVFSCSVMHEALHNHYTQKSLSLSLGGGGGSGGGGSAPAPAPAPAPAPAPAPAPAPGGGGSGGGGSDHCPLGPGRCCRLHTVRASLEDLGWADWVLSPREVQVTMCIGACPSQFRAANMHAQIKTSLHRLKPDTVPAPCCVPASYNPMVLIQKTDTGVSLQTYDDLLAKDCHCI

SEQ ID NO: 97 - protein, 359 aa, synthetic construct
GGPSVFLFPPKPKDTLMISRTPEVTCVVVDVSQEDPEVQFNWYVDGVEVHNAKTKPREEQFNSTYRVVSVLTVLHQDWLNGKEYKCKVSNKGLPSSIEKTISKAKGQPREPQVYTLPPSQEEMTKNQVSLTCLVKGFYPSDIAVEWESNGQPENNYKTTPPVLDSDGSFFLYSRLTVDKSRWQEGNVFSCSVMHEALHNHYTQESLSLSLGGGGGSGGGGSAPAPAPAPAPAPAPAPAPAPGGGGSGGGGSDHCPLGPGRCCRLHTVRASLEDLGWADWVLSPREVQVTMCIGACPSQFRAANMHAQIKTSLHRLKPDTVPAPCCVPASYNPMVLIQKTDTGVSLQTYDDLLAKDCHCI

SEQ ID NO: 98 - protein, 358 aa, synthetic construct
GPSVFLFPPKPKDTLMISRTPEVTCVVVDVSQEDPEVQFNWYVDGVEVHNAKTKPREEQFNSTYRVVSVLTVLHQDWLNGKEYKCKVSNKGLPSSIEKTISKAKGQPREPQVYTLPPSQEEMTKNQVSLTCLVKGFYPSDIAVEWESNGQPENNYKTTPPVLDSDGSFFLYSRLTVDKSRWQEGNVFSCSVMHEALHNHYTQESLSLSLGGGGGSGGGGSAPAPAPAPAPAPAPAPAPAPGGGGSGGGGSDHCPLGPGRCCRLHTVRASLEDLGWADWVLSPREVQVTMCIGACPSQFRAANMHAQIKTSLHRLKPDTVPAPCCVPASYNPMVLIQKTDTGVSLQTYDDLLAKDCHCI

SEQ ID NO: 99 - protein, 348 aa, synthetic construct
GGPSVFLFPPKPKDTLMISRTPEVTCVVVDVSQEDPEVQFNWYVDGVEVHNAKTKPREEQFNSTYRVVSVLTVLHQDWLNGKEYKCKVSNKGLPSSIEKTISKAKGQPREPQVYTLPPSQEEMTKNQVSLTCLVKGFYPSDIAVEWESNGQPENNYKTTPPVLDSDGSFFLYSRLTVDKSRWQEGNVFSCSVMHEALHNHYTQESLSLSLGGGGGAPAPAPAPAPAPAPAPAPAPGGGGGDHCPLGPGRCCRLHTVRASLEDLGWADWVLSPREVQVTMCIGACPSQFRAANMHAQIKTSLHRLKPDTVPAPCCVPASYNPMVLIQKTDTGVSLQTYDDLLAKDCHCI

SEQ ID NO: 100 - protein, 359 aa, synthetic construct
GGPSVFLFPPKPKDTLMISRTPEVTCVVVDVSQEDPEVQFNWYVDGVEVHNAKTKPREEQFNSTYRVVSVLTVLHQDWLNGKEYKCKVSNKGLPSSIEKTISKAKGQPREPQVYTLPPSQEEMTKNQVSLTCLVKGFYPSDIAVEWESNGQPENNYKTTPPVLDSDGSFFLYSRLTVDKSRWQEGNVFSCSVMHEALHNHYTQESLSLSLGGGGGSGGGGSEPEPEPEPEPEPEPEPEPEPGGGGSGGGGSDHCPLGPGRCCRLHTVRASLEDLGWADWVLSPREVQVTMCIGACPSQFRAANMHAQIKTSLHRLKPDTVPAPCCVPASYNPMVLIQKTDTGVSLQTYDDLLAKDCHCI

SEQ ID NO: 101 - protein, 359 aa, synthetic construct
GGPSVFLFPPKPKDTLMISRTPEVTCVVVDVSQEDPEVQFNWYVDGVEVHNAKTKPREEQFNSTYRVVSVLTVLHQDWLNGKEYKCKVSNKGLPSSIEKTISKAKGQPREPQVYTLPPSQEEMTKNQVSLTCLVKGFYPSDIAVEWESNGQPENNYKTTPPVLDSDGSFFLYSRLTVDKSRWQEGNVFSCSVMHEALHNHYTQESLSLSLGGGGGSGGGGSGGGGSGGGGSGGGGSGGGGSGGGGSGGGGSDHCPLGPGRCCRLHTVRASLEDLGWADWVLSPREVQVTMCIGACPSQFRAANMHAQIKTSLHRLKPDTVPAPCCVPASYNPMVLIQKTDTGVSLQTYDDLLAKDCHCI

SEQ ID NO: 102 - protein, 364 aa, synthetic construct
APEAAGGPSVFLFPPKPKDTLMISRTPEVTCVVVDVSQEDPEVQFNWYVDGVEVHNAKTKPREEQFNSTYRVVSVLTVLHQDWLNGKEYKCKVSNKGLPSSIEKTISKAKGQPREPQVYTLPPSQEEMTKNQVSLTCLVKGFYPSDIAVEWESNGQPENNYKTTPPVLDSDGSFFLYSRLTVDKSRWQEGNVFSCSVMHEALHNHYTQESLSLSLGGGGGSGGGGSAPAPAPAPAPAPAPAPAPAPGGGGSGGGGSEHCPLGPGRCCRLHTVRASLEDLGWADWVLSPREVQVTMCIGACPSQFRAANMHAQIKTSLHRLKPDTVPAPCCVPASYNPMVLIQKTDTGVSLQTYDDLLAKDCHCI

SEQ ID NO: 103 - protein, 363 aa, synthetic construct
APEAAGGPSVFLFPPKPKDTLMISRTPEVTCVVVDVSQEDPEVQFNWYVDGVEVHNAKTKPREEQFNSTYRVVSVLTVLHQDWLNGKEYKCKVSNKGLPSSIEKTISKAKGQPREPQVYTLPPSQEEMTKNQVSLTCLVKGFYPSDIAVEWESNGQPENNYKTTPPVLDSDGSFFLYSRLTVDKSRWQEGNVFSCSVMHEALHNHYTQESLSLSLGGGGGSGGGGSAPAPAPAPAPAPAPAPAPAPGGGGSGGGGSDCPLGPGRCCRLHTVRASLEDLGWADWVLSPREVQVTMCIGACPSQFRAANMHAQIKTSLHRLKPDTVPAPCCVPASYNPMVLIQKTDTGVSLQTYDDLLAKDCHCI

SEQ ID NO: 104 - protein, 364 aa, synthetic construct
APEAAGGPSVFLFPPKPKDTLMISRTPEVTCVVVDVSQEDPEVQFNWYVDGVEVHNAKTKPREEQFNSTYRVVSVLTVLHQDWLNGKEYKCKVSNKGLPSSIEKTISKAKGQPREPQVYTLPPSQEEMTKNQVSLTCLVKGFYPSDIAVEWESNGQPENNYKTTPPVLDSDGSFFLYSRLTVDKSRWQEGNVFSCSVMHEALHNHYTQESLSLSLGGGGGSGGGGSAPAPAPAPAPAPAPAPAPAPGGGGSGGGGSDECPLGPGRCCRLHTVRASLEDLGWADWVLSPREVQVTMCIGACPSQFRAANMHAQIKTSLHRLKPDTVPAPCCVPASYNPMVLIQKTDTGVSLQTYDDLLAKDCHCI

SEQ ID NO: 105 - protein, 363 aa, synthetic construct
APEAAGGPSVFLFPPKPKDTLMISRTPEVTCVVVDVSQEDPEVQFNWYVDGVEVHNAKTKPREEQFNSTYRVVSVLTVLHQDWLNGKEYKCKVSNKGLPSSIEKTISKAKGQPREPQVYTLPPSQEEMTKNQVSLTCLVKGFYPSDIAVEWESNGQPENNYKTTPPVLDSDGSFFLYSRLTVDKSRWQEGNVFSCSVMHEALHNHYTQESLSLSLGGGGGSGGGGSAPAPAPAPAPAPAPAPAPAPGGGGSGGGGSECPLGPGRCCRLHTVRASLEDLGWADWVLSPREVQVTMCIGACPSQFRAANMHAQIKTSLHRLKPDTVPAPCCVPASYNPMVLIQKTDTGVSLQTYDDLLAKDCHCI

SEQ ID NO: 106 - protein, 364 aa, synthetic construct
APEAAGGPSVFLFPPKPKDTLMISRTPEVTCVVVDVSQEDPEVQFNWYVDGVEVHNAKTKPREEQFNSTYRVVSVLTVLHQDWLNGKEYKCKVSNKGLPSSIEKTISKAKGQPREPQVYTLPPSQEEMTKNQVSLTCLVKGFYPSDIAVEWESNGQPENNYKTTPPVLDSDGSFFLYSRLTVDKSRWQEGNVFSCSVMHEALHNHYTQESLSLSLGGGGGSGGGGSAPAPAPAPAPAPAPAPAPAPGGGGSGGGGSDHCPLGPGRCCRLHTVQASLEDLGWADWVLSPREVQVTMCIGACPSQFRAANMHAQIKTSLHRLKPDTVPAPCCVPASYNPMVLIQKTDTGVSLQTYDDLLAKDCHCI

SEQ ID NO: 107 - protein, 364 aa, synthetic construct
APEAAGGPSVFLFPPKPKDTLMISRTPEVTCVVVDVSQEDPEVQFNWYVDGVEVHNAKTKPREEQFNSTYRVVSVLTVLHQDWLNGKEYKCKVSNKGLPSSIEKTISKAKGQPREPQVYTLPPSQEEMTKNQVSLTCLVKGFYPSDIAVEWESNGQPENNYKTTPPVLDSDGSFFLYSRLTVDKSRWQEGNVFSCSVMHEALHNHYTQESLSLSLGGGGGSGGGGSAPAPAPAPAPAPAPAPAPAPGGGGSGGGGSDHCPLGPGRCCRLHTVHASLEDLGWADWVLSPREVQVTMCIGACPSQFRAANMHAQIKTSLHRLKPDTVPAPCCVPASYNPMVLIQKTDTGVSLQTYDDLLAKDCHCI

SEQ ID NO: 108 - protein, 364 aa, synthetic construct
APEAAGGPSVFLFPPKPKDTLMISRTPEVTCVVVDVSQEDPEVQFNWYVDGVEVHNAKTKPREEQFNSTYRVVSVLTVLHQDWLNGKEYKCKVSNKGLPSSIEKTISKAKGQPREPQVYTLPPSQEEMTKNQVSLTCLVKGFYPSDIAVEWESNGQPENNYKTTPPVLDSDGSFFLYSRLTVDKSRWQEGNVFSCSVMHEALHNHYTQESLSLSLGGGGGSGGGGSAPAPAPAPAPAPAPAPAPAPGGGGSGGGGSDHCPLGPGRCCRLHTVRASLEELGWADWVLSPREVQVTMCIGACPSQFRAANMHAQIKTSLHRLKPDTVPAPCCVPASYNPMVLIQKTDTGVSLQTYDDLLAKDCHCI

SEQ ID NO: 109 - protein, 364 aa, synthetic construct
APEAAGGPSVFLFPPKPKDTLMISRTPEVTCVVVDVSQEDPEVQFNWYVDGVEVHNAKTKPREEQFNSTYRVVSVLTVLHQDWLNGKEYKCKVSNKGLPSSIEKTISKAKGQPREPQVYTLPPSQEEMTKNQVSLTCLVKGFYPSDIAVEWESNGQPENNYKTTPPVLDSDGSFFLYSRLTVDKSRWQEGNVFSCSVMHEALHNHYTQESLSLSLGGGGGSGGGGSAPAPAPAPAPAPAPAPAPAPGGGGSGGGGSDHCPLGPGRCCRLHTVRASLEELGWADWVLSPREVQVTMCIGACPSQFRAANMHAQIKTSLHRLRPDTVPAPCCVPASYNPMVLIQKTDTGVSLQTYDDLLAKDCHCI

SEQ ID NO: 110 - protein, 364 aa, synthetic construct; identical to SEQ ID NO: 86

SEQ ID NO: 111 - protein, 364 aa, synthetic construct
APEAAGGPSVFLFPPKPKDTLMISRTPEVTCVVVDVSQEDPEVQFNWYVDGVEVHNAKTKPREEQFNSTYRVVSVLTVLHQDWLNGKEYKCKVSNKGLPSSIEKTISKAKGQPREPQVYTLPPSQEEMTKNQVSLTCLVKGFYPSDIAVEWESNGQPENNYKTTPPVLDSDGSFFLYSRLTVDKSRWQEGNVFSCSVMHEALHNHYTQESLSLSLGGGGGSGGGGSAPAPAPAPAPAPAPAPAPAPGGGGSGGGGSDHCPLGPGRCCRLHTVRASLEDLGWADWVLSPREVQVTMCIGDCPSQFRAANMHAQIKTSLHRLKPDTVPAPCCVPASYNPMVLIQKTDTGVSLQTYDDLLAKDCHCI

SEQ ID NO: 112 - protein, 364 aa, synthetic construct
APEAAGGPSVFLFPPKPKDTLMISRTPEVTCVVVDVSQEDPEVQFNWYVDGVEVHNAKTKPREEQFNSTYRVVSVLTVLHQDWLNGKEYKCKVSNKGLPSSIEKTISKAKGQPREPQVYTLPPSQEEMTKNQVSLTCLVKGFYPSDIAVEWESNGQPENNYKTTPPVLDSDGSFFLYSRLTVDKSRWQEGNVFSCSVMHEALHNHYTQESLSLSLGGGGGSGGGGSAPAPAPAPAPAPAPAPAPAPGGGGSGGGGSDHCPLGPGRCCRLHTVRASLEDLGWADWVLSPREVQVTMCIGACPSQFRSANMHAQIKTSLHRLKPDTVPAPCCVPASYNPMVLIQKTDTGVSLQTYDDLLAKDCHCI

SEQ ID NO: 113 - protein, 364 aa, synthetic construct
APEAAGGPSVFLFPPKPKDTLMISRTPEVTCVVVDVSQEDPEVQFNWYVDGVEVHNAKTKPREEQFNSTYRVVSVLTVLHQDWLNGKEYKCKVSNKGLPSSIEKTISKAKGQPREPQVYTLPPSQEEMTKNQVSLTCLVKGFYPSDIAVEWESNGQPENNYKTTPPVLDSDGSFFLYSRLTVDKSRWQEGNVFSCSVMHEALHNHYTQESLSLSLGGGGGSGGGGSAPAPAPAPAPAPAPAPAPAPGGGGSGGGGSDHCPLGPGRCCRLHTVRASLEDLGWADWVLSPREVQVTMCIGACPSQFRAENMHAQIKTSLHRLKPDTVPAPCCVPASYNPMVLIQKTDTGVSLQTYDDLLAKDCHCI

SEQ ID NO: 114 - protein, 364 aa, synthetic construct
APEAAGGPSVFLFPPKPKDTLMISRTPEVTCVVVDVSQEDPEVQFNWYVDGVEVHNAKTKPREEQFNSTYRVVSVLTVLHQDWLNGKEYKCKVSNKGLPSSIEKTISKAKGQPREPQVYTLPPSQEEMTKNQVSLTCLVKGFYPSDIAVEWESNGQPENNYKTTPPVLDSDGSFFLYSRLTVDKSRWQEGNVFSCSVMHEALHNHYTQESLSLSLGGGGGSGGGGSAPAPAPAPAPAPAPAPAPAPGGGGSGGGGSDHCPLGPGRCCRLHTVRASLEDLGWADWVLSPREVQVTMCIGACPSQFRAANTHAQIKTSLHRLKPDTVPAPCCVPASYNPMVLIQKTDTGVSLQTYDDLLAKDCHCI

SEQ ID NO: 115 - protein, 364 aa, synthetic construct
APEAAGGPSVFLFPPKPKDTLMISRTPEVTCVVVDVSQEDPEVQFNWYVDGVEVHNAKTKPREEQFNSTYRVVSVLTVLHQDWLNGKEYKCKVSNKGLPSSIEKTISKAKGQPREPQVYTLPPSQEEMTKNQVSLTCLVKGFYPSDIAVEWESNGQPENNYKTTPPVLDSDGSFFLYSRLTVDKSRWQEGNVFSCSVMHEALHNHYTQESLSLSLGGGGGSGGGGSAPAPAPAPAPAPAPAPAPAPGGGGSGGGGSDHCPLGPGRCCRLHTVRASLEDLGWADWVLSPREVQVTMCIGACPSQFRAANMHAQIKTSLHQLKPDTVPAPCCVPASYNPMVLIQKTDTGVSLQTYDDLLAKDCHCI

SEQ ID NO: 116 - protein, 364 aa, synthetic construct
APEAAGGPSVFLFPPKPKDTLMISRTPEVTCVVVDVSQEDPEVQFNWYVDGVEVHNAKTKPREEQFNSTYRVVSVLTVLHQDWLNGKEYKCKVSNKGLPSSIEKTISKAKGQPREPQVYTLPPSQEEMTKNQVSLTCLVKGFYPSDIAVEWESNGQPENNYKTTPPVLDSDGSFFLYSRLTVDKSRWQEGNVFSCSVMHEALHNHYTQESLSLSLGGGGGSGGGGSAPAPAPAPAPAPAPAPAPAPGGGGSGGGGSDHCPLGPGRCCRLHTVRASLEDLGWADWVLSPREVQVTMCIGACPSQFRAANMHAQIKTSLHRLKPDTVPAPCCVPSSYNPMVLIQKTDTGVSLQTYDDLLAKDCHCI

SEQ ID NO: 117 - protein, 364 aa, synthetic construct
APEAAGGPSVFLFPPKPKDTLMISRTPEVTCVVVDVSQEDPEVQFNWYVDGVEVHNAKTKPREEQFNSTYRVVSVLTVLHQDWLNGKEYKCKVSNKGLPSSIEKTISKAKGQPREPQVYTLPPSQEEMTKNQVSLTCLVKGFYPSDIAVEWESNGQPENNYKTTPPVLDSDGSFFLYSRLTVDKSRWQEGNVFSCSVMHEALHNHYTQESLSLSLGGGGGSGGGGSAPAPAPAPAPAPAPAPAPAPGGGGSGGGGSDHCPLGPGRCCRLHTVRASLEDLGWADWVLSPREVQVTMCIGACPSQFRAANMHAQIKTSLHRLKPDTVPAPCCVPASYNPMVLIQKTDEGVSLQTYDDLLAKDCHCI

SEQ ID NO: 118 - protein, 364 aa, synthetic construct
APEAAGGPSVFLFPPKPKDTLMISRTPEVTCVVVDVSQEDPEVQFNWYVDGVEVHNAKTKPREEQFNSTYRVVSVLTVLHQDWLNGKEYKCKVSNKGLPSSIEKTISKAKGQPREPQVYTLPPSQEEMTKNQVSLTCLVKGFYPSDIAVEWESNGQPENNYKTTPPVLDSDGSFFLYSRLTVDKSRWQEGNVFSCSVMHEALHNHYTQESLSLSLGGGGGSGGGGSAPAPAPAPAPAPAPAPAPAPGGGGSGGGGSDHCPLGPGRCCRLHTVRASLEDLGWADWVLSPREVQVTMCIGACPSQFRAANMHAQIKTSLHRLKPDTVPAPCCVPASYNPMVLIQKTDTGVSLQTYDDLLAQDCHCI

SEQ ID NO: 119 - protein, 354 aa, synthetic construct
APEAAGGPSVFLFPPKPKDTLMISRTPEVTCVVVDVSQEDPEVQFNWYVDGVEVHNAKTKPREEQFNSTYRVVSVLTVLHQDWLNGKEYKCKVSNKGLPSSIEKTISKAKGQPREPQVYTLPPSQEEMTKNQVSLTCLVKGFYPSDIAVEWESNGQPENNYKTTPPVLDSDGSFFLYSRLTVDKSRWQEGNVFSCSVMHEALHNHYTQESLSLSLGGGGGSGGGGSAPAPAPAPAPAPAPAPAPAPGGGGSGGGGSCRLHTVRASLEDLGWADWVLSPREVQVTMCIGACPSQFRAANMHAQIKTSLHRLKPDTVPAPCCVPASYNPMVLIQKTDTGVSLQTYDDLLAKDCHCI

SEQ ID NO: 120 - protein, 365 aa, synthetic construct
APEAAGGPSVFLFPPKPKDTLMISRTPEVTCVVVDVSQEDPEVQFNWYVDGVEVHNAKTKPREEQFNSTYRVVSVLTVLHQDWLNGKEYKCKVSNKGLPSSIEKTISKAKGQPREPQVYTLPPSQEEMTKNQVSLTCLVKGFYPSDIAVEWESNGQPENNYKTTPPVLDSDGSFFLYSRLTVDKSRWQEGNVFSCSVMHEALHNHYTQQSLSLSLGGGGGSGGGGSAPAPAPAPAPAPAPAPAPAPGGGGSGGGGSGDHCPLGPGRCCRLHTVRASLEDLGWADWVLSPREVQVTMCIGACPSQFRAANMHAQIKTSLHRLKPDTVPAPCCVPASYNPMVLIQKTDTGVSLQTYDDLLAKDCHCI

SEQ ID NO: 121 - protein, 365 aa, synthetic construct
APEAAGGPSVFLFPPKPKDTLMISRTPEVTCVVVDVSQEDPEVQFNWYVDGVEVHNAKTKPREEQFNSTYRVVSVLTVLHQDWLNGKEYKCKVSNKGLPSSIEKTISKAKGQPREPQVYTLPPSQQEMTKNQVSLTCLVKGFYPSDIAVEWESNGQPENNYKTTPPVLDSDGSFFLYSRLTVDKSRWQEGNVFSCSVMHEALHNHYTQKSLSLSLGGGGGSGGGGSAPAPAPAPAPAPAPAPAPAPGGGGSGGGGSGDHCPLGPGRCCRLHTVRASLEDLGWADWVLSPREVQVTMCIGACPSQFRAANMHAQIKTSLHRLKPDTVPAPCCVPASYNPMVLIQKTDTGVSLQTYDDLLAKDCHCI

SEQ ID NO: 122 - protein, 365 aa, synthetic construct
APEAAGGPSVFLFPPKPKDTLMISRTPEVTCVVVDVSQEDPEVQFNWYVDGVEVHNAKTKPREEQFNSTYRVVSVLTVLHQDWLNGKEYKCKVSNKGLPSSIEKTISKAKGQPREPQVYTLPPSQEEMTKNQVSLTCLVKGFYPSDIAVEWESNGQPENNYKTTPPVLDSDGSFFLYSRLTVDKSRWQEGNVFSCSVMHEALHNHYTQNSLSLSLGGGGGSGGGGSAPAPAPAPAPAPAPAPAPAPGGGGSGGGGSGDHCPLGPGRCCRLHTVRASLEDLGWADWVLSPREVQVTMCIGACPSQFRAANMHAQIKTSLHRLKPDTVPAPCCVPASYNPMVLIQKTDTGVSLQTYDDLLAKDCHCI

SEQ ID NO: 123 - protein, 365 aa, synthetic construct
APEAAGGPSVFLFPPKPKDTLMISRTPEVTCVVVDVSQEDPEVQFNWYVDGVEVHNAKTKPREEQFNSTYRVVSVLTVLHQDWLNGKEYKCKVSNKGLPSSIEKTISKAKGQPREPQVYTLPPSQNEMTKNQVSLTCLVKGFYPSDIAVEWESNGQPENNYKTTPPVLDSDGSFFLYSRLTVDKSRWQEGNVFSCSVMHEALHNHYTQKSLSLSLGGGGGSGGGGSAPAPAPAPAPAPAPAPAPAPGGGGSGGGGSGDHCPLGPGRCCRLHTVRASLEDLGWADWVLSPREVQVTMCIGACPSQFRAANMHAQIKTSLHRLKPDTVPAPCCVPASYNPMVLIQKTDTGVSLQTYDDLLAKDCHCI

SEQ ID NO: 124 - protein, 365 aa, synthetic construct
APEAAGGPSVFLFPPKPKDTLMISRTPEVTCVVVDVSQEDPEVQFNWYVDGVEVHNAKTKPREEQFNSTYRVVSVLTVLHQDWLNGKEYKCKVSNKGLPSSIEKTISKAKGQPREPQVYTLPPSQEEMTKNQVSLTCLVKGFYPSDIAVEWESNGQPENNYKTTPPVLDSDGSFFLYSRLTVDKSRWQEGNVFSCSVMHEALHNHYTQASLSLSLGGGGGSGGGGSAPAPAPAPAPAPAPAPAPAPGGGGSGGGGSGDHCPLGPGRCCRLHTVRASLEDLGWADWVLSPREVQVTMCIGACPSQFRAANMHAQIKTSLHRLKPDTVPAPCCVPASYNPMVLIQKTDTGVSLQTYDDLLAKDCHCI

SEQ ID NO: 125 - protein, 365 aa, synthetic construct
APEAAGGPSVFLFPPKPKDTLMISRTPEVTCVVVDVSQEDPEVQFNWYVDGVEVHNAKTKPREEQFNSTYRVVSVLTVLHQDWLNGKEYKCKVSNKGLPSSIEKTISKAKGQPREPQVYTLPPSQAEMTKNQVSLTCLVKGFYPSDIAVEWESNGQPENNYKTTPPVLDSDGSFFLYSRLTVDKSRWQEGNVFSCSVMHEALHNHYTQKSLSLSLGGGGGSGGGGSAPAPAPAPAPAPAPAPAPAPGGGGSGGGGSGDHCPLGPGRCCRLHTVRASLEDLGWADWVLSPREVQVTMCIGACPSQFRAANMHAQIKTSLHRLKPDTVPAPCCVPASYNPMVLIQKTDTGVSLQTYDDLLAKDCHCI

SEQ ID NO: 126 - protein, 363 aa, synthetic construct
APEAAGGPSVFLFPPKPKDTLMISRTPEVTCVVVDVSQEDPEVQFNWYVDGVEVHNAKTKPREEQFNSTYRVVSVLTVLHQDWLNGKEYKCKVSNKGLPSSIEKTISKAKGQPREPQVYTLPPSQEEMTKNQVSLTCLVKGFYPSDIAVEWESNGQPENNYKTTPPVLDSDGSFFLYSRLTVDKSRWQEGNVFSCSVMHEALHNHYTQQSLSLSLGGGGGAGGGGAPAPAPAPAPAPAPAPAPAPGGGGAGGGGGDHCPLGPGRCCRLHTVRASLEDLGWADWVLSPREVQVTMCIGACPSQFRAANMHAQIKTSLHRLKPDTVPAPCCVPASYNPMVLIQKTDTGVSLQTYDDLLAKDCHCI

SEQ ID NO: 127 - protein, 363 aa, synthetic construct
APEAAGGPSVFLFPPKPKDTLMISRTPEVTCVVVDVSQEDPEVQFNWYVDGVEVHNAKTKPREEQFNSTYRVVSVLTVLHQDWLNGKEYKCKVSNKGLPSSIEKTISKAKGQPREPQVYTLPPSQEEMTKNQVSLTCLVKGFYPSDIAVEWESNGQPENNYKTTPPVLDSDGSFFLYSRLTVDKSRWQEGNVFSCSVMHEALHNHYTQESLSLSLGGGGGAGGGGAPAPAPAPAPAPAPAPAPAPGGGGAGGGGGDHCPLGPGRCCRLHTVRASLEDLGWADWVLSPREVQVTMCIGACPSQFRAANMHAQIKTSLHRLKPDTVPAPCCVPASYNPMVLIQKTDTGVSLQTYDDLLAKDCHCI

SEQ ID NO: 128 - protein, 365 aa, synthetic construct
APEAAGGPSVFLFPPKPKDTLMISRTPEVTCVVVDVSQEDPEVQFNWYVDGVEVHNAKTKPREEQFNSTYRVVSVLTVLHQDWLNGKEYKCKVSNKGLPSSIEKTISKAKGQPREPQVYTLPPSQEEMTKNQVSLTCLVKGFYPSDIAVEWESNGQPENNYKTTPPVLDSDGSFFLYSRLTVDKSRWQEGNVFSCSVMHEALHNHYTQDSLSLSLGGGGGSGGGGSAPAPAPAPAPAPAPAPAPAPGGGGSGGGGSGDHCPLGPGRCCRLHTVRASLEDLGWADWVLSPREVQVTMCIGACPSQFRAANMHAQIKTSLHRLKPDTVPAPCCVPASYNPMVLIQKTDTGVSLQTYDDLLAKDCHCI

SEQ ID NO: 129 - protein, 365 aa, synthetic construct
APEAAGGPSVFLFPPKPKDTLMISRTPEVTCVVVDVSQEDPEVQFNWYVDGVEVHNAKTKPREEQFNSTYRVVSVLTVLHQDWLNGKEYKCKVSNKGLPSSIEKTISKAKGQPREPQVYTLPPSQKEMTKNQVSLTCLVKGFYPSDIAVEWESNGQPENNYKTTPPVLDSDGSFFLYSRLTVDKSRWQEGNVFSCSVMHEALHNHYTQKSLSLSLGGGGGSGGGGSAPAPAPAPAPAPAPAPAPAPGGGGSGGGGSGDHCPLGPGRCCRLHTVRASLEDLGWADWVLSPREVQVTMCIGACPSQFRAANMHAQIKTSLHRLKPDTVPAPCCVPASYNPMVLIQKTDTGVSLQTYDDLLAKDCHCI

SEQ ID NO: 130 - protein, 365 aa, synthetic construct
APEAAGGPSVFLFPPKPKDTLMISRTPEVTCVVVDVSQEDPEVQFNWYVDGVEVHNAKTKPREEQFNSTYRVVSVLTVLHQDWLNGKEYKCKVSNKGLPSSIEKTISKAKGQPREPQVYTLPPSQREMTKNQVSLTCLVKGFYPSDIAVEWESNGQPENNYKTTPPVLDSDGSFFLYSRLTVDKSRWQEGNVFSCSVMHEALHNHYTQKSLSLSLGGGGGSGGGGSAPAPAPAPAPAPAPAPAPAPGGGGSGGGGSGDHCPLGPGRCCRLHTVRASLEDLGWADWVLSPREVQVTMCIGACPSQFRAANMHAQIKTSLHRLKPDTVPAPCCVPASYNPMVLIQKTDTGVSLQTYDDLLAKDCHCI